European Patent Application EP 4 570 894 A2, published June 18, 2025. Title: MANNANASE VARIANTS AND POLYNUCLEOTIDES ENCODING SAME. Applicant: Novozymes A/S. The sequence listing filed with the application follows.

SEQUENCE LISTING (4 sequences)

SEQ ID NO: 1 - protein, 326 aa, Bacillus bogoriensis
MKQQKRLYARLLTLLFALIFLLPHSAAAANSGFYVSGTTLYDANGNPFVMRGINHGHAWYKDQATTAIEGIANTGANTVRIVLSDGGQWTKDDIHTVRNLISLAEDNHLVAVLEVHDATGYDSIASLNRAVDYWIEMRSALIGKEDTVIINIANEWFGSWEGDAWADGYKQAIPRLRNAGLNHTLMVDAAGWGQFPQSIHDYGREVFNADPQRNTMFSIHMYEYAGGNASQVRTNIDRVLNQDLALVIGEFGHRHTNGDVDEATIMSYSEQRGVGWLAWSWKGNGPEWEYLDLSNDWAGNNLTAWGNTIVNGPYGLRETSRLSTVF

SEQ ID NO: 2 - protein, 298 aa, Bacillus bogoriensis
ANSGFYVSGTTLYDANGNPFVMRGINHGHAWYKDQATTAIEGIANTGANTVRIVLSDGGQWTKDDIHTVRNLISLAEDNHLVAVLEVHDATGYDSIASLNRAVDYWIEMRSALIGKEDTVIINIANEWFGSWEGDAWADGYKQAIPRLRNAGLNHTLMVDAAGWGQFPQSIHDYGREVFNADPQRNTMFSIHMYEYAGGNASQVRTNIDRVLNQDLALVIGEFGHRHTNGDVDEATIMSYSEQRGVGWLAWSWKGNGPEWEYLDLSNDWAGNNLTAWGNTIVNGPYGLRETSRLSTVF

SEQ ID NO: 3 - DNA, 981 bp, Bacillus bogoriensis
  source 1..981: mol_type = unassigned DNA
atgaaacaacaaaaacggctttacgcccgattgctgacgctgttatttgcgctcatcttcttgctgcctcattctgcagccgcggcaaattccggattttatgtaagcggtaccactctatacgatgccaatggaaacccatttgtaatgagagggattaaccatgggcacgcatggtataaagaccaggcaactactgcaattgaagggattgcaaataccggtgctaatacggtccggattgtgttatctgatgggggacaatggacaaaagatgacatccatacagtaagaaaccttatctctttagcggaagataatcatttggttgctgttcttgaagttcatgatgctaccggttatgattccattgcttcgctcaatcgtgctgttgattattggattgaaatgagaagtgctttaattggaaaggaagataccgtcattattaatattgcgaatgaatggtttggttcgtgggaaggggatgcttgggctgacgggtataaacaagcaatcccgcgattgcgtaacgccggtctaaaccataccttgatggtagatgctgcggggtggggacaatttccacaatcgattcatgattatggaagagaagtttttaatgctgaccctcaacgaaatacaatgttttcgattcatatgtatgaatatgcaggtggtaatgcatcgcaagttcgtactaatattgaccgagttcttaatcaagacctcgcattagtcattggtgaatttggacaccgtcatacaaatggtgacgtcgatgaagcaacgattatgagctattctgaacaaagaggagttgggtggttggcgtggtcatggaaagggaacggcccagaatgggagtatttagacctttcgaatgattgggctggaaataaccttacagcttggggaaatacaatagtgaatggtccatatggtttaagagaaacttcgagattaagcaccgttttttga

SEQ ID NO: 4 - protein, 269 aa, Bacillus subtilis
AQSVPWGISRVQAPAAHNRGLTGSGVKVAVLDTGISTHPDLNIRGGASFVPGEPSTQDGNGHGTHVAGTIAALNNSIGVLGVAPSAELYAVKVLGASGSGSVSSIAQGLEWAGNNGMHVANLSLGSPSPSATLEQAVNSATSRGVLVVAASGNSGAGSISYPARYANAMAVGATDQNNNRASFSQYGAGLDIVAPGVNVQSTYPGSTYASLNGTSMATPHVAGAAALVKQKNPSWSNVQIRNHLKNTATSLGSTNLYGSGLVNAEAATR